European Patent Specification EP 3 826 720 B1, published April 22, 2026. Title: Nucleic acids for inhibiting expression of TMPRSS6 and iron chelators. Applicant: Silence Therapeutics GmbH. The sequence listing filed with the application follows.

SEQUENCE LISTING (449 sequences)

SEQ ID NO: 1 - RNA, 19 nt, Artificial Sequence
  siRNA
  modified_base, modified as per summary sequence table at the end of the description
augucuuucacacuggcuu

SEQ ID NO: 2 - RNA, 19 nt, Artificial Sequence
  siRNA
  modified_base, modified as per summary sequence table at the end of the description
aagccagugugaaagacau

SEQ ID NO: 3 - RNA, 19 nt, Artificial Sequence
  siRNA
  modified_base, modified as per summary sequence table at the end of the description
auugaguacacgcagacug

SEQ ID NO: 4 - RNA, 19 nt, Artificial Sequence
  siRNA
  modified_base, modified as per summary sequence table at the end of the description
cagucugcguguacucaau

SEQ ID NO: 5 - RNA, 19 nt, Artificial Sequence
  siRNA
  modified_base, modified as per summary sequence table at the end of the description
aaguugauggugaucccgg

SEQ ID NO: 6 - RNA, 19 nt, Artificial Sequence
  siRNA
  modified_base, modified as per summary sequence table at the end of the description
ccgggaucaccaucaacuu

SEQ ID NO: 7 - RNA, 19 nt, Artificial Sequence
  siRNA
  modified_base, modified as per summary sequence table at the end of the description
uucuggaucguccacuggc

SEQ ID NO: 8 - RNA, 19 nt, Artificial Sequence
  siRNA
  modified_base, modified as per summary sequence table at the end of the description
gccaguggacgauccagaa

SEQ ID NO: 9 - RNA, 19 nt, Artificial Sequence
  siRNA
  modified_base, modified as per summary sequence table at the end of the description
auucacagaacagaggaac

SEQ ID NO: 10 - RNA, 19 nt, Artificial Sequence
  siRNA
  modified_base, modified as per summary sequence table at the end of the description
guuccucuguucugugaau

SEQ ID NO: 11 - RNA, 19 nt, Artificial Sequence
  siRNA
  modified_base, modified as per summary sequence table at the end of the description
guagucauggcuguccucu

SEQ ID NO: 12 - RNA, 19 nt, Artificial Sequence
  siRNA
  modified_base, modified as per summary sequence table at the end of the description
agaggacagccaugacuac

SEQ ID NO: 13 - RNA, 19 nt, Artificial Sequence
  siRNA
  modified_base, modified as per summary sequence table at the end of the description
aguuguaguaaguucccag

SEQ ID NO: 14 - RNA, 19 nt, Artificial Sequence
  siRNA
  modified_base, modified as per summary sequence table at the end of the description
cugggaacuuacuacaacu

SEQ ID NO: 15 - RNA, 19 nt, Artificial Sequence
  siRNA
  modified_base, modified as per summary sequence table at the end of the description
uuguacccuaggaaauacc

SEQ ID NO: 16 - RNA, 19 nt, Artificial Sequence
  siRNA
  modified_base, modified as per summary sequence table at the end of the description
gguauuuccuaggguacaa

SEQ ID NO: 17 - RNA, 19 nt, Artificial Sequence
  siRNA
  modified_base, modified as per summary sequence table at the end of the description
aaccagaagaagcagguga

SEQ ID NO: 18 - RNA, 19 nt, Artificial Sequence
  siRNA
  modified_base, modified as per summary sequence table at the end of the description
ucaccugcuucuucugguu

SEQ ID NO: 19 - RNA, 19 nt, Artificial Sequence
  siRNA
  modified_base, modified as per summary sequence table at the end of the description
uaacaacccagcguggaau

SEQ ID NO: 20 - RNA, 19 nt, Artificial Sequence
  siRNA
  modified_base, modified as per summary sequence table at the end of the description
auuccacgcuggguuguua

SEQ ID NO: 21 - RNA, 19 nt, Artificial Sequence
  siRNA
  modified_base, modified as per summary sequence table at the end of the description
guuucucucauccaggccg

SEQ ID NO: 22 - RNA, 19 nt, Artificial Sequence
  siRNA
  modified_base, modified as per summary sequence table at the end of the description
cggccuggaugagagaaac

SEQ ID NO: 23 - RNA, 19 nt, Artificial Sequence
  siRNA
  modified_base, modified as per summary sequence table at the end of the description
gcaucuucugggcuuuggc

SEQ ID NO: 24 - RNA, 19 nt, Artificial Sequence
  siRNA
  modified_base, modified as per summary sequence table at the end of the description
gccaaagcccagaagaugc

SEQ ID NO: 25 - RNA, 19 nt, Artificial Sequence
  siRNA
  modified_base, modified as per summary sequence table at the end of the description
ucacacuggaaggugaaug

SEQ ID NO: 26 - RNA, 19 nt, Artificial Sequence
  siRNA
  modified_base, modified as per summary sequence table at the end of the description
cauucaccuuccaguguga

SEQ ID NO: 27 - RNA, 19 nt, Artificial Sequence
  siRNA
  modified_base, modified as per summary sequence table at the end of the description
cacagaugugucgaccccg

SEQ ID NO: 28 - RNA, 19 nt, Artificial Sequence
  siRNA
  modified_base, modified as per summary sequence table at the end of the description
cggggucgacacaucugug

SEQ ID NO: 29 - RNA, 19 nt, Artificial Sequence
  siRNA
  modified_base, modified as per summary sequence table at the end of the description
uguacccuaggaaauacca

SEQ ID NO: 30 - RNA, 19 nt, Artificial Sequence
  siRNA
  modified_base, modified as per summary sequence table at the end of the description
ugguauuuccuaggguaca

SEQ ID NO: 31 - RNA, 19 nt, Artificial Sequence
  siRNA
  modified_base, modified as per summary sequence table at the end of the description
ucgaaguauuccgcguacg

SEQ ID NO: 32 - RNA, 19 nt, Artificial Sequence
  siRNA
  modified_base, modified as per summary sequence table at the end of the description
cguacgcggaauacuucga

SEQ ID NO: 33 - RNA, 19 nt, Artificial Sequence
  siRNA
  modified_base, modified as per summary sequence table at the end of the description
uaaguucuagcuguggugg

SEQ ID NO: 34 - RNA, 19 nt, Artificial Sequence
  siRNA
  modified_base, modified as per summary sequence table at the end of the description
ccaccacagcuagaacuua

SEQ ID NO: 35 - RNA, 17 nt, Artificial Sequence
  siRNA
ccgccaaagcccagaag

SEQ ID NO: 36 - RNA, 21 nt, Artificial Sequence
  siRNA
ggtccctccccaaaggaatag

SEQ ID NO: 37 - RNA, 28 nt, Artificial Sequence
  siRNA
cagcacccgcctgggaacttactacaac

SEQ ID NO: 38 - RNA, 21 nt, Artificial Sequence
  siRNA
cggcacctaccttccactctt

SEQ ID NO: 39 - RNA, 17 nt, Artificial Sequence
  siRNA
tcggtggtgggcatcct

SEQ ID NO: 40 - RNA, 28 nt, Artificial Sequence
  siRNA
ccgagatgtttccagctcccctgttcta

SEQ ID NO: 41 - RNA, 23 nt, Artificial Sequence
  siRNA
gcatgggtcagaaggattcctat

SEQ ID NO: 42 - RNA, 23 nt, Artificial Sequence
  siRNA
tgtagaaggtgtggtgccagatt

SEQ ID NO: 43 - RNA, 22 nt, Artificial Sequence
  siRNA
tcgagcacggcatcgtcaccaa

SEQ ID NO: 44 - RNA, 22 nt, Artificial Sequence
  siRNA
gtttgagaccttcaacacccca

SEQ ID NO: 45 - RNA, 21 nt, Artificial Sequence
  siRNA
gaccagaggcatacagggaca

SEQ ID NO: 46 - RNA, 26 nt, Artificial Sequence
  siRNA
ccatgtacgtagccatccaggctgtg

SEQ ID NO: 47 - RNA, 22 nt, Artificial Sequence
  siRNA
caccgccaaatttaactgcaga

SEQ ID NO: 48 - RNA, 24 nt, Artificial Sequence
  siRNA
aagggtttgataagttctagctgt

SEQ ID NO: 49 - RNA, 31 nt, Artificial Sequence
  siRNA
tgcacagtatccttttgaagaccataaccca

SEQ ID NO: 50 - RNA, 22 nt, Artificial Sequence
  siRNA
cctgtctcctgcttctcctcct

SEQ ID NO: 51 - RNA, 22 nt, Artificial Sequence
  siRNA
aatgtctgccctgctttcttcc

SEQ ID NO: 52 - RNA, 28 nt, Artificial Sequence
  siRNA
tgagcagcaccacctatctccatcaaca

SEQ ID NO: 53 - RNA, 19 nt, Artificial Sequence
  siRNA
  modified_base, modified as per summary sequence table at the end of the description
gguauuuccuaggguacaa

SEQ ID NO: 54 - RNA, 19 nt, Artificial Sequence
  siRNA
  modified_base, modified as per summary sequence table at the end of the description
cagucugcguguacucaau

SEQ ID NO: 55 - RNA, 19 nt, Artificial Sequence
  siRNA
  modified_base, modified as per summary sequence table at the end of the description
gccaaagcccagaagaugc

SEQ ID NO: 56 - RNA, 19 nt, Artificial Sequence
  siRNA
  modified_base, modified as per summary sequence table at the end of the description
cugggaacuuacuacaacu

SEQ ID NO: 57 - RNA, 19 nt, Artificial Sequence
  siRNA
  modified_base, modified as per summary sequence table at the end of the description
ucaccugcuucuucugguu

SEQ ID NO: 58 - RNA, 19 nt, Artificial Sequence
  siRNA
  modified_base, modified as per summary sequence table at the end of the description
aagccagugugaaagacau

SEQ ID NO: 59 - RNA, 19 nt, Artificial Sequence
  siRNA
  modified_base, modified as per summary sequence table at the end of the description
auuccacgcuggguuguua

SEQ ID NO: 60 - RNA, 19 nt, Artificial Sequence
  siRNA
  modified_base, modified as per summary sequence table at the end of the description
gccaguggacgauccagaa

SEQ ID NO: 61 - RNA, 19 nt, Artificial Sequence
  siRNA
  modified_base, modified as per summary sequence table at the end of the description
ccgggaucaccaucaacuu

SEQ ID NO: 62 - RNA, 19 nt, Artificial Sequence
  siRNA
  modified_base, modified as per summary sequence table at the end of the description
guuccucuguucugugaau

SEQ ID NO: 63 - RNA, 19 nt, Artificial Sequence
  siRNA
  modified_base, modified as per summary sequence table at the end of the description
cggccuggaugagagaaac

SEQ ID NO: 64 - RNA, 19 nt, Artificial Sequence
  siRNA
  modified_base, modified as per summary sequence table at the end of the description
cauucaccuuccaguguga

SEQ ID NO: 65 - RNA, 19 nt, Artificial Sequence
  siRNA
  modified_base, modified as per summary sequence table at the end of the description
cggggucgacacaucugug

SEQ ID NO: 66 - RNA, 19 nt, Artificial Sequence
  siRNA
  modified_base, modified as per summary sequence table at the end of the description
agaggacagccaugacuac

SEQ ID NO: 67 - RNA, 19 nt, Artificial Sequence
  siRNA
  modified_base, modified as per summary sequence table at the end of the description
aaccagaagaagcagguga

SEQ ID NO: 68 - RNA, 19 nt, Artificial Sequence
  siRNA
  modified_base, modified as per summary sequence table at the end of the description
ucaccugcuucuucugguu

SEQ ID NO: 69 - RNA, 19 nt, Artificial Sequence
  siRNA
  modified_base, modified as per summary sequence table at the end of the description
aaccagaagaagcagguga

SEQ ID NO: 70 - RNA, 19 nt, Artificial Sequence
  siRNA
  modified_base, modified as per summary sequence table at the end of the description
ucaccugcuucuucugguu

SEQ ID NO: 71 - RNA, 19 nt, Artificial Sequence
  siRNA
  modified_base, modified as per summary sequence table at the end of the description
aaccagaagaagcagguga

SEQ ID NO: 72 - RNA, 19 nt, Artificial Sequence
  siRNA
  modified_base, modified as per summary sequence table at the end of the description
ucaccugcuucuucugguu

SEQ ID NO: 73 - RNA, 19 nt, Artificial Sequence
  siRNA
  modified_base, modified as per summary sequence table at the end of the description
aaccagaagaagcagguga

SEQ ID NO: 74 - RNA, 19 nt, Artificial Sequence
  siRNA
  modified_base, modified as per summary sequence table at the end of the description
aaccagaagaagcagguga

SEQ ID NO: 75 - RNA, 19 nt, Artificial Sequence
  siRNA
  modified_base, modified as per summary sequence table at the end of the description
ucaccugcuucuucugguu

SEQ ID NO: 76 - RNA, 19 nt, Artificial Sequence
  siRNA
  modified_base, modified as per summary sequence table at the end of the description
aaccagaagaagcagguga

SEQ ID NO: 77 - RNA, 19 nt, Artificial Sequence
  siRNA
  modified_base, modified as per summary sequence table at the end of the description
aaccagaagaagcagguga

SEQ ID NO: 78 - RNA, 19 nt, Artificial Sequence
  siRNA
  modified_base, modified as per summary sequence table at the end of the description
aaccagaagaagcagguga

SEQ ID NO: 79 - RNA, 19 nt, Artificial Sequence
  siRNA
  modified_base, modified as per summary sequence table at the end of the description
aaccagaagaagcagguga

SEQ ID NO: 80 - RNA, 19 nt, Artificial Sequence
  siRNA
  modified_base, modified as per summary sequence table at the end of the description
aaccagaagaagcagguga

SEQ ID NO: 81 - RNA, 19 nt, Artificial Sequence
  siRNA
  modified_base, modified as per summary sequence table at the end of the description
aaccagaagaagcagguga

SEQ ID NO: 82 - RNA, 19 nt, Artificial Sequence
  siRNA
  modified_base, modified as per summary sequence table at the end of the description
aaccagaagaagcagguga

SEQ ID NO: 83 - RNA, 19 nt, Artificial Sequence
  siRNA
  modified_base, modified as per summary sequence table at the end of the description
aaccagaagaagcagguga

SEQ ID NO: 84 - RNA, 19 nt, Artificial Sequence
  siRNA
  modified_base, modified as per summary sequence table at the end of the description
ucaccugcuucuucugguu

SEQ ID NO: 85 - RNA, 19 nt, Artificial Sequence
  siRNA
  modified_base, modified as per summary sequence table at the end of the description
aaccagaagaagcagguga

SEQ ID NO: 86 - RNA, 19 nt, Artificial Sequence
  siRNA
  modified_base, modified as per summary sequence table at the end of the description
ucaccugcuucuucugguu

SEQ ID NO: 87 - RNA, 19 nt, Artificial Sequence
  siRNA
  modified_base, modified as per summary sequence table at the end of the description
aaccagaagaagcagguga

SEQ ID NO: 88 - RNA, 19 nt, Artificial Sequence
  siRNA
  modified_base, modified as per summary sequence table at the end of the description
aaccagaagaagcagguga

SEQ ID NO: 89 - RNA, 19 nt, Artificial Sequence
  siRNA
  modified_base, modified as per summary sequence table at the end of the description
ucaccugcuucuucugguu

SEQ ID NO: 90 - RNA, 19 nt, Artificial Sequence
  siRNA
  modified_base, modified as per summary sequence table at the end of the description
aaccagaagaagcagguga

SEQ ID NO: 91 - RNA, 19 nt, Artificial Sequence
  siRNA
  modified_base, modified as per summary sequence table at the end of the description
aaccagaagaagcagguga

SEQ ID NO: 92 - RNA, 19 nt, Artificial Sequence
  siRNA
  modified_base, modified as per summary sequence table at the end of the description
aaccagaagaagcagguga

SEQ ID NO: 93 - RNA, 19 nt, Artificial Sequence
  siRNA
  modified_base, modified as per summary sequence table at the end of the description
aaccagaagaagcagguga

SEQ ID NO: 94 - RNA, 19 nt, Artificial Sequence
  siRNA
  modified_base, modified as per summary sequence table at the end of the description
aaccagaagaagcagguga

SEQ ID NO: 95 - RNA, 19 nt, Artificial Sequence
  siRNA
  modified_base, modified as per summary sequence table at the end of the description
aaccagaagaagcagguga

SEQ ID NO: 96 - RNA, 19 nt, Artificial Sequence
  siRNA
  modified_base, modified as per summary sequence table at the end of the description
aaccagaagaagcagguga

SEQ ID NO: 97 - RNA, 19 nt, Artificial Sequence
  siRNA
  modified_base, modified as per summary sequence table at the end of the description
aaccagaagaagcagguga

SEQ ID NO: 98 - RNA, 19 nt, Artificial Sequence
  siRNA
  modified_base, modified as per summary sequence table at the end of the description
aaccagaagaagcagguga

SEQ ID NO: 99 - RNA, 19 nt, Artificial Sequence
  siRNA
  modified_base, modified as per summary sequence table at the end of the description
aaccagaagaagcagguga

SEQ ID NO: 100 - RNA, 19 nt, Artificial Sequence
  siRNA
  modified_base, modified as per summary sequence table at the end of the description
ucaccugcuucuucugguu

SEQ ID NO: 101 - RNA, 19 nt, Artificial Sequence
  siRNA
  modified_base, modified as per summary sequence table at the end of the description
ucaccugcuucuucugguu

SEQ ID NO: 102 - RNA, 19 nt, Artificial Sequence
  siRNA
  modified_base, modified as per summary sequence table at the end of the description
ucaccugcuucuucugguu

SEQ ID NO: 103 - RNA, 19 nt, Artificial Sequence
  siRNA
  modified_base, modified as per summary sequence table at the end of the description
ucaccugcuucuucugguu

SEQ ID NO: 104 - RNA, 19 nt, Artificial Sequence
  siRNA
  modified_base, modified as per summary sequence table at the end of the description
ucaccugcuucuucugguu

SEQ ID NO: 105 - RNA, 19 nt, Artificial Sequence
  siRNA
  modified_base, modified as per summary sequence table at the end of the description
ucaccugcuucuucugguu

SEQ ID NO: 106 - RNA, 19 nt, Artificial Sequence
  siRNA
  modified_base, modified as per summary sequence table at the end of the description
ucaccugcuucuucugguu

SEQ ID NO: 107 - RNA, 21 nt, Artificial Sequence
  siRNA
  modified_base, modified as per summary sequence table at the end of the description
ucuugguuacaugaaauccca

SEQ ID NO: 108 - RNA, 21 nt, Artificial Sequence
  siRNA
  modified_base, modified as per summary sequence table at the end of the description
ugggauuucauguaaccaaga

SEQ ID NO: 109 - RNA, 19 nt, Artificial Sequence
  siRNA
  modified_base, modified as per summary sequence table at the end of the description
ucgaaguauuccgcguacg

SEQ ID NO: 110 - RNA, 19 nt, Artificial Sequence
  siRNA
  modified_base, modified as per summary sequence table at the end of the description
cguacgcggaauacuucga

SEQ ID NO: 111 - RNA, 19 nt, Artificial Sequence
  siRNA
  modified_base, modified as per summary sequence table at the end of the description
aaccagaagaagcagguga

SEQ ID NO: 112 - RNA, 19 nt, Artificial Sequence
  siRNA
  modified_base, modified as per summary sequence table at the end of the description
ucaccugcuucuucugguu

SEQ ID NO: 113 - RNA, 19 nt, Artificial Sequence
  siRNA
  modified_base, modified as per summary sequence table at the end of the description
aaccagaagaagcagguga

SEQ ID NO: 114 - RNA, 19 nt, Artificial Sequence
  siRNA
  modified_base, modified as per summary sequence table at the end of the description
ucaccugcuucuucugguu

SEQ ID NO: 115 - RNA, 19 nt, Artificial Sequence
  siRNA
  modified_base, modified as per summary sequence table at the end of the description
aaccagaagaagcagguga

SEQ ID NO: 116 - RNA, 19 nt, Artificial Sequence
  siRNA
  modified_base, modified as per summary sequence table at the end of the description
ucaccugcuucuucugguu

SEQ ID NO: 117 - RNA, 19 nt, Artificial Sequence
  siRNA
  modified_base, modified as per summary sequence table at the end of the description
aaccagaagaagcagguga

SEQ ID NO: 118 - DNA, 19 bp, Artificial Sequence
  /note="combined DNA/RNA molecule" /note="siRNA"
  modified_base, modified as per summary sequence table at the end of the description
ucaccugcuucuucuggut

SEQ ID NO: 119 - RNA, 19 nt, Artificial Sequence
  siRNA
  modified_base, modified as per summary sequence table at the end of the description
aaccagaagaagcagguga

SEQ ID NO: 120 - RNA, 19 nt, Artificial Sequence
  siRNA
  modified_base, modified as per summary sequence table at the end of the description
ucaccugcuucuucugguu

SEQ ID NO: 121 - RNA, 19 nt, Artificial Sequence
  siRNA
  modified_base, modified as per summary sequence table at the end of the description
aaccagaagaagcagguga

SEQ ID NO: 122 - RNA, 19 nt, Artificial Sequence
  siRNA
  modified_base, modified as per summary sequence table at the end of the description
ucaccugcuucuucugguu

SEQ ID NO: 123 - RNA, 21 nt, Artificial Sequence
  siRNA
  modified_base, modified as per summary sequence table at the end of the description
aaccagaagaagcaggugacc

SEQ ID NO: 124 - RNA, 19 nt, Artificial Sequence
  siRNA
  modified_base, modified as per summary sequence table at the end of the description
ucaccugcuucuucugguu

SEQ ID NO: 125 - RNA, 19 nt, Artificial Sequence
  siRNA
  modified_base, modified as per summary sequence table at the end of the description
aaccagaagaagcagguga

SEQ ID NO: 126 - RNA, 19 nt, Artificial Sequence
  siRNA
  modified_base, modified as per summary sequence table at the end of the description
ucaccugcuucuucugguu

SEQ ID NO: 127 - RNA, 19 nt, Artificial Sequence
  siRNA
  modified_base, modified as per summary sequence table at the end of the description
aaccagaagaagcagguga

SEQ ID NO: 128 - RNA, 19 nt, Artificial Sequence
  siRNA
  modified_base, modified as per summary sequence table at the end of the description
ucaccugcuucuucugguu

SEQ ID NO: 129 - RNA, 19 nt, Artificial Sequence
  siRNA
  modified_base, modified as per summary sequence table at the end of the description
aaccagaagaagcagguga

SEQ ID NO: 130 - RNA, 19 nt, Artificial Sequence
  siRNA
  modified_base, modified as per summary sequence table at the end of the description
ucaccugcuucuucugguu

SEQ ID NO: 131 - RNA, 19 nt, Artificial Sequence
  siRNA
  modified_base, modified as per summary sequence table at the end of the description
uuaguaaaccuuuugagac

SEQ ID NO: 132 - RNA, 19 nt, Artificial Sequence
  siRNA
  modified_base, modified as per summary sequence table at the end of the description
gucucaaaagguuuacuaa

SEQ ID NO: 133 - RNA, 19 nt, Artificial Sequence
  siRNA
  modified_base, modified as per summary sequence table at the end of the description
cugaggacgcccugggagu

SEQ ID NO: 134 - RNA, 19 nt, Artificial Sequence
  siRNA
  modified_base, modified as per summary sequence table at the end of the description
acucccagggcguccucag

SEQ ID NO: 135 - RNA, 19 nt, Artificial Sequence
  siRNA
  modified_base, modified as per summary sequence table at the end of the description
gcugaggacgcccugggag

SEQ ID NO: 136 - RNA, 19 nt, Artificial Sequence
  siRNA
  modified_base, modified as per summary sequence table at the end of the description
cucccagggcguccucagc

SEQ ID NO: 137 - RNA, 19 nt, Artificial Sequence
  siRNA
  modified_base, modified as per summary sequence table at the end of the description
ugcugaggacgcccuggga

SEQ ID NO: 138 - RNA, 19 nt, Artificial Sequence
  siRNA
  modified_base, modified as per summary sequence table at the end of the description
ucccagggcguccucagca

SEQ ID NO: 139 - RNA, 19 nt, Artificial Sequence
  siRNA
  modified_base, modified as per summary sequence table at the end of the description
gugcugaggacgcccuggg

SEQ ID NO: 140 - RNA, 19 nt, Artificial Sequence
  siRNA
  modified_base, modified as per summary sequence table at the end of the description
cccagggcguccucagcac

SEQ ID NO: 141 - RNA, 19 nt, Artificial Sequence
  siRNA
  modified_base, modified as per summary sequence table at the end of the description
ggugcugaggacgcccugg

SEQ ID NO: 142 - RNA, 19 nt, Artificial Sequence
  siRNA
  modified_base, modified as per summary sequence table at the end of the description
ccagggcguccucagcacc

SEQ ID NO: 143 - RNA, 19 nt, Artificial Sequence
  siRNA
  modified_base, modified as per summary sequence table at the end of the description
gggugcugaggacgcccug

SEQ ID NO: 144 - RNA, 19 nt, Artificial Sequence
  siRNA
  modified_base, modified as per summary sequence table at the end of the description
cagggcguccucagcaccc

SEQ ID NO: 145 - RNA, 19 nt, Artificial Sequence
  siRNA
  modified_base, modified as per summary sequence table at the end of the description
cggggugcugaggacgccc

SEQ ID NO: 146 - RNA, 19 nt, Artificial Sequence
  siRNA
  modified_base, modified as per summary sequence table at the end of the description
gggcguccucagcaccccg

SEQ ID NO: 147 - RNA, 19 nt, Artificial Sequence
  siRNA
  modified_base, modified as per summary sequence table at the end of the description
acggggugcugaggacgcc

SEQ ID NO: 148 - RNA, 19 nt, Artificial Sequence
  siRNA
  modified_base, modified as per summary sequence table at the end of the description
ggcguccucagcaccccgu

SEQ ID NO: 149 - RNA, 19 nt, Artificial Sequence
  siRNA
  modified_base, modified as per summary sequence table at the end of the description
uacggggugcugaggacgc

SEQ ID NO: 150 - RNA, 19 nt, Artificial Sequence
  siRNA
  modified_base, modified as per summary sequence table at the end of the description
gcguccucagcaccccgua

SEQ ID NO: 151 - RNA, 19 nt, Artificial Sequence
  siRNA
  modified_base, modified as per summary sequence table at the end of the description
guacggggugcugaggacg

SEQ ID NO: 152 - RNA, 19 nt, Artificial Sequence
  siRNA
  modified_base, modified as per summary sequence table at the end of the description
cguccucagcaccccguac

SEQ ID NO: 153 - RNA, 19 nt, Artificial Sequence
  siRNA
  modified_base, modified as per summary sequence table at the end of the description
aguacggggugcugaggac

SEQ ID NO: 154 - RNA, 19 nt, Artificial Sequence
  siRNA
  modified_base, modified as per summary sequence table at the end of the description
guccucagcaccccguacu

SEQ ID NO: 155 - RNA, 19 nt, Artificial Sequence
  siRNA
  modified_base, modified as per summary sequence table at the end of the description
aaguacggggugcugagga

SEQ ID NO: 156 - RNA, 19 nt, Artificial Sequence
  siRNA
  modified_base, modified as per summary sequence table at the end of the description
uccucagcaccccguacuu

SEQ ID NO: 157 - RNA, 19 nt, Artificial Sequence
  siRNA
  modified_base, modified as per summary sequence table at the end of the description
ggaaguacggggugcugag

SEQ ID NO: 158 - RNA, 19 nt, Artificial Sequence
  siRNA
  modified_base, modified as per summary sequence table at the end of the description
cucagcaccccguacuucc

SEQ ID NO: 159 - RNA, 19 nt, Artificial Sequence
  siRNA
  modified_base, modified as per summary sequence table at the end of the description
gggaaguacggggugcuga

SEQ ID NO: 160 - RNA, 19 nt, Artificial Sequence
  siRNA
  modified_base, modified as per summary sequence table at the end of the description
ucagcaccccguacuuccc

SEQ ID NO: 161 - RNA, 19 nt, Artificial Sequence
  siRNA
  modified_base, modified as per summary sequence table at the end of the description
ggggaaguacggggugcug

SEQ ID NO: 162 - RNA, 19 nt, Artificial Sequence
  siRNA
  modified_base, modified as per summary sequence table at the end of the description
cagcaccccguacuucccc

SEQ ID NO: 163 - RNA, 19 nt, Artificial Sequence
  siRNA
  modified_base, modified as per summary sequence table at the end of the description
uggggaaguacggggugcu

SEQ ID NO: 164 - RNA, 19 nt, Artificial Sequence
  siRNA
  modified_base, modified as per summary sequence table at the end of the description
agcaccccguacuucccca

SEQ ID NO: 165 - RNA, 19 nt, Artificial Sequence
  siRNA
  modified_base, modified as per summary sequence table at the end of the description
cuggggaaguacggggugc

SEQ ID NO: 166 - RNA, 19 nt, Artificial Sequence
  siRNA
  modified_base, modified as per summary sequence table at the end of the description
gcaccccguacuuccccag

SEQ ID NO: 167 - RNA, 19 nt, Artificial Sequence
  siRNA
  modified_base, modified as per summary sequence table at the end of the description
agcuggggaaguacggggu

SEQ ID NO: 168 - RNA, 19 nt, Artificial Sequence
  siRNA
  modified_base, modified as per summary sequence table at the end of the description
accccguacuuccccagcu

SEQ ID NO: 169 - RNA, 19 nt, Artificial Sequence
  siRNA
  modified_base, modified as per summary sequence table at the end of the description
uagcuggggaaguacgggg

SEQ ID NO: 170 - RNA, 19 nt, Artificial Sequence
  siRNA
  modified_base, modified as per summary sequence table at the end of the description
ccccguacuuccccagcua

SEQ ID NO: 171 - RNA, 19 nt, Artificial Sequence
  siRNA
  modified_base, modified as per summary sequence table at the end of the description
guagcuggggaaguacggg

SEQ ID NO: 172 - RNA, 19 nt, Artificial Sequence
  siRNA
  modified_base, modified as per summary sequence table at the end of the description
cccguacuuccccagcuac

SEQ ID NO: 173 - RNA, 19 nt, Artificial Sequence
  siRNA
  modified_base, modified as per summary sequence table at the end of the description
aguagcuggggaaguacgg

SEQ ID NO: 174 - RNA, 19 nt, Artificial Sequence
  siRNA
  modified_base, modified as per summary sequence table at the end of the description
ccguacuuccccagcuacu

SEQ ID NO: 175 - RNA, 19 nt, Artificial Sequence
  siRNA
  modified_base, modified as per summary sequence table at the end of the description
guaguagcuggggaaguac

SEQ ID NO: 176 - RNA, 19 nt, Artificial Sequence
  siRNA
  modified_base, modified as per summary sequence table at the end of the description
guacuuccccagcuacuac

SEQ ID NO: 177 - RNA, 19 nt, Artificial Sequence
  siRNA
  modified_base, modified as per summary sequence table at the end of the description
aguaguagcuggggaagua

SEQ ID NO: 178 - RNA, 19 nt, Artificial Sequence
  siRNA
  modified_base, modified as per summary sequence table at the end of the description
uacuuccccagcuacuacu

SEQ ID NO: 179 - RNA, 19 nt, Artificial Sequence
  siRNA
  modified_base, modified as per summary sequence table at the end of the description
gaguaguagcuggggaagu

SEQ ID NO: 180 - RNA, 19 nt, Artificial Sequence
  siRNA
  modified_base, modified as per summary sequence table at the end of the description
acuuccccagcuacuacuc

SEQ ID NO: 181 - RNA, 19 nt, Artificial Sequence
  siRNA
  modified_base, modified as per summary sequence table at the end of the description
cgaguaguagcuggggaag

SEQ ID NO: 182 - RNA, 19 nt, Artificial Sequence
  siRNA
  modified_base, modified as per summary sequence table at the end of the description
cuuccccagcuacuacucg

SEQ ID NO: 183 - RNA, 19 nt, Artificial Sequence
  siRNA
  modified_base, modified as per summary sequence table at the end of the description
gcgaguaguagcuggggaa

SEQ ID NO: 184 - RNA, 19 nt, Artificial Sequence
  siRNA
  modified_base, modified as per summary sequence table at the end of the description
uuccccagcuacuacucgc

SEQ ID NO: 185 - RNA, 19 nt, Artificial Sequence
  siRNA
  modified_base, modified as per summary sequence table at the end of the description
ggcgaguaguagcugggga

SEQ ID NO: 186 - RNA, 19 nt, Artificial Sequence
  siRNA
  modified_base, modified as per summary sequence table at the end of the description
uccccagcuacuacucgcc

SEQ ID NO: 187 - RNA, 19 nt, Artificial Sequence
  siRNA
  modified_base, modified as per summary sequence table at the end of the description
gggcgaguaguagcugggg

SEQ ID NO: 188 - RNA, 19 nt, Artificial Sequence
  siRNA
  modified_base, modified as per summary sequence table at the end of the description
ccccagcuacuacucgccc

SEQ ID NO: 189 - RNA, 19 nt, Artificial Sequence
  siRNA
  modified_base, modified as per summary sequence table at the end of the description
ggggcgaguaguagcuggg

SEQ ID NO: 190 - RNA, 19 nt, Artificial Sequence
  siRNA
  modified_base, modified as per summary sequence table at the end of the description
cccagcuacuacucgcccc

SEQ ID NO: 191 - RNA, 19 nt, Artificial Sequence
  siRNA
  modified_base, modified as per summary sequence table at the end of the description
uggggcgaguaguagcugg

SEQ ID NO: 192 - RNA, 19 nt, Artificial Sequence
  siRNA
  modified_base, modified as per summary sequence table at the end of the description
ccagcuacuacucgcccca

SEQ ID NO: 193 - RNA, 19 nt, Artificial Sequence
  siRNA
  modified_base, modified as per summary sequence table at the end of the description
uuggggcgaguaguagcug

SEQ ID NO: 194 - RNA, 19 nt, Artificial Sequence
  siRNA
  modified_base, modified as per summary sequence table at the end of the description
cagcuacuacucgccccaa

SEQ ID NO: 195 - RNA, 19 nt, Artificial Sequence
  siRNA
  modified_base, modified as per summary sequence table at the end of the description
uauuccaaagggcagcuga

SEQ ID NO: 196 - RNA, 19 nt, Artificial Sequence
  siRNA
  modified_base, modified as per summary sequence table at the end of the description
ucagcugcccuuuggaaua

SEQ ID NO: 197 - RNA, 19 nt, Artificial Sequence
  siRNA
  modified_base, modified as per summary sequence table at the end of the description
aucuucugggcuuuggcgg

SEQ ID NO: 198 - RNA, 19 nt, Artificial Sequence
  siRNA
  modified_base, modified as per summary sequence table at the end of the description
ccgccaaagcccagaagau

SEQ ID NO: 199 - RNA, 19 nt, Artificial Sequence
  siRNA
  modified_base, modified as per summary sequence table at the end of the description
uuuucucuuggaguccuca

SEQ ID NO: 200 - RNA, 19 nt, Artificial Sequence
  siRNA
  modified_base, modified as per summary sequence table at the end of the description
ugaggacuccaagagaaaa

SEQ ID NO: 201 - RNA, 19 nt, Artificial Sequence
  siRNA
  modified_base, modified as per summary sequence table at the end of the description
gaauagacggagcuggagu

SEQ ID NO: 202 - RNA, 19 nt, Artificial Sequence
  siRNA
  modified_base, modified as per summary sequence table at the end of the description
acuccagcuccgucuauuc

SEQ ID NO: 203 - RNA, 19 nt, Artificial Sequence
  siRNA
  modified_base, modified as per summary sequence table at the end of the description
uaguagcuggggaaguacg

SEQ ID NO: 204 - RNA, 19 nt, Artificial Sequence
  siRNA
  modified_base, modified as per summary sequence table at the end of the description
cguacuuccccagcuacua

SEQ ID NO: 205 - RNA, 19 nt, Artificial Sequence
  siRNA
  modified_base, modified as per summary sequence table at the end of the description
agauccugggagaaguggc

SEQ ID NO: 206 - RNA, 19 nt, Artificial Sequence
  siRNA
  modified_base, modified as per summary sequence table at the end of the description
gccacuucucccaggaucu

SEQ ID NO: 207 - RNA, 19 nt, Artificial Sequence
  siRNA
  modified_base, modified as per summary sequence table at the end of the description
cuguucuggaucguccacu

SEQ ID NO: 208 - RNA, 19 nt, Artificial Sequence
  siRNA
  modified_base, modified as per summary sequence table at the end of the description
aguggacgauccagaacag

SEQ ID NO: 209 - RNA, 19 nt, Artificial Sequence
  siRNA
  modified_base, modified as per summary sequence table at the end of the description
cucaccuugaaggacaccu

SEQ ID NO: 210 - RNA, 19 nt, Artificial Sequence
  siRNA
  modified_base, modified as per summary sequence table at the end of the description
agguguccuucaaggugag

SEQ ID NO: 211 - RNA, 19 nt, Artificial Sequence
  siRNA
  modified_base, modified as per summary sequence table at the end of the description
aguuucucucauccaggcc

SEQ ID NO: 212 - RNA, 19 nt, Artificial Sequence
  siRNA
  modified_base, modified as per summary sequence table at the end of the description
ggccuggaugagagaaacu

SEQ ID NO: 213 - RNA, 19 nt, Artificial Sequence
  siRNA
  modified_base, modified as per summary sequence table at the end of the description
guacccuaggaaauaccag

SEQ ID NO: 214 - RNA, 19 nt, Artificial Sequence
  siRNA
  modified_base, modified as per summary sequence table at the end of the description
cugguauuuccuaggguac

SEQ ID NO: 215 - RNA, 19 nt, Artificial Sequence
  siRNA
  modified_base, modified as per summary sequence table at the end of the description
cuguugacuguggacagca

SEQ ID NO: 216 - RNA, 19 nt, Artificial Sequence
  siRNA
  modified_base, modified as per summary sequence table at the end of the description
ugcuguccacagucaacag

SEQ ID NO: 217 - RNA, 19 nt, Artificial Sequence
  siRNA
  modified_base, modified as per summary sequence table at the end of the description
aaccagaagaagcagguga

SEQ ID NO: 218 - RNA, 19 nt, Artificial Sequence
  siRNA
  modified_base, modified as per summary sequence table at the end of the description
ucaccugcuucuucugguu

SEQ ID NO: 219 - RNA, 19 nt, Artificial Sequence
  siRNA
  modified_base, modified as per summary sequence table at the end of the description
aaccagaagaagcagguga

SEQ ID NO: 220 - RNA, 19 nt, Artificial Sequence
  siRNA
  modified_base, modified as per summary sequence table at the end of the description
ucaccugcuucuucugguu

SEQ ID NO: 221 - RNA, 19 nt, Artificial Sequence
  siRNA
  modified_base, modified as per summary sequence table at the end of the description
aaccagaagaagcagguga

SEQ ID NO: 222 - RNA, 19 nt, Artificial Sequence
  siRNA
  modified_base, modified as per summary sequence table at the end of the description
ucaccugcuucuucugguu

SEQ ID NO: 223 - RNA, 19 nt, Artificial Sequence
  siRNA
  modified_base, modified as per summary sequence table at the end of the description
ucgaaguauuccgcguacg

SEQ ID NO: 224 - RNA, 19 nt, Artificial Sequence
  siRNA
  modified_base, modified as per summary sequence table at the end of the description
cguacgcggaauacuucga

SEQ ID NO: 225 - RNA, 19 nt, Artificial Sequence
  siRNA
  modified_base, modified as per summary sequence table at the end of the description
aaccagaagaagcagguga

SEQ ID NO: 226 - RNA, 19 nt, Artificial Sequence
  siRNA
  modified_base, modified as per summary sequence table at the end of the description
ucaccugcuucuucugguu

SEQ ID NO: 227 - RNA, 19 nt, Artificial Sequence
  siRNA
  modified_base, modified as per summary sequence table at the end of the description
aaccagaagaagcagguga

SEQ ID NO: 228 - RNA, 19 nt, Artificial Sequence
  siRNA
  modified_base, modified as per summary sequence table at the end of the description
ucaccugcuucuucugguu

SEQ ID NO: 229 - RNA, 19 nt, Artificial Sequence
  siRNA
  modified_base, modified as per summary sequence table at the end of the description
aaccagaagaagcagguga

SEQ ID NO: 230 - RNA, 19 nt, Artificial Sequence
  siRNA
  modified_base, modified as per summary sequence table at the end of the description
ucaccugcuucuucugguu

SEQ ID NO: 231 - RNA, 19 nt, Artificial Sequence
  siRNA
  modified_base, modified as per summary sequence table at the end of the description
aaccagaagaagcagguga

SEQ ID NO: 232 - RNA, 19 nt, Artificial Sequence
  siRNA
  modified_base, modified as per summary sequence table at the end of the description
ucaccugcuucuucugguu

SEQ ID NO: 233 - RNA, 19 nt, Artificial Sequence
  siRNA
  modified_base, modified as per summary sequence table at the end of the description
aaccagaagaagcagguga

SEQ ID NO: 234 - RNA, 19 nt, Artificial Sequence
  siRNA
  modified_base, modified as per summary sequence table at the end of the description
ucaccugcuucuucugguu

SEQ ID NO: 235 - RNA, 19 nt, Artificial Sequence
  siRNA
  modified_base, modified as per summary sequence table at the end of the description
aaccagaagaagcagguga

SEQ ID NO: 236 - RNA, 19 nt, Artificial Sequence
  siRNA
  modified_base, modified as per summary sequence table at the end of the description
ucaccugcuucuucugguu

SEQ ID NO: 237 - RNA, 19 nt, Artificial Sequence
  siRNA
  modified_base, modified as per summary sequence table at the end of the description
aaccagaagaagcagguga

SEQ ID NO: 238 - RNA, 19 nt, Artificial Sequence
  siRNA
  modified_base, modified as per summary sequence table at the end of the description
ucaccugcuucuucugguu

SEQ ID NO: 239 - RNA, 19 nt, Artificial Sequence
  siRNA
  modified_base, modified as per summary sequence table at the end of the description
aaccagaagaagcagguga

SEQ ID NO: 240 - RNA, 19 nt, Artificial Sequence
  siRNA
  modified_base, modified as per summary sequence table at the end of the description
ucaccugcuucuucugguu

SEQ ID NO: 241 - RNA, 19 nt, Artificial Sequence
  siRNA
  modified_base, modified as per summary sequence table at the end of the description
aaccagaagaagcagguga

SEQ ID NO: 242 - RNA, 19 nt, Artificial Sequence
  siRNA
  modified_base, modified as per summary sequence table at the end of the description
ucaccugcuucuucugguu

SEQ ID NO: 243 - RNA, 19 nt, Artificial Sequence
  siRNA
  modified_base, modified as per summary sequence table at the end of the description
aaccagaagaagcagguga

SEQ ID NO: 244 - RNA, 19 nt, Artificial Sequence
  siRNA
  modified_base, modified as per summary sequence table at the end of the description
ucaccugcuucuucugguu

SEQ ID NO: 245 - RNA, 19 nt, Artificial Sequence
  siRNA
  modified_base, modified as per summary sequence table at the end of the description
aaccagaagaagcagguga

SEQ ID NO: 246 - RNA, 19 nt, Artificial Sequence
  siRNA
  modified_base, modified as per summary sequence table at the end of the description
ucaccugcuucuucugguu

SEQ ID NO: 247 - RNA, 19 nt, Artificial Sequence
  siRNA
  modified_base, modified as per summary sequence table at the end of the description
aaccagaagaagcagguga

SEQ ID NO: 248 - RNA, 19 nt, Artificial Sequence
  siRNA
  modified_base, modified as per summary sequence table at the end of the description
ucaccugcuucuucugguu

SEQ ID NO: 249 - RNA, 19 nt, Artificial Sequence
  siRNA
  modified_base, modified as per summary sequence table at the end of the description
aaccagaagaagcagguga

SEQ ID NO: 250 - RNA, 19 nt, Artificial Sequence
  siRNA
  modified_base, modified as per summary sequence table at the end of the description
ucaccugcuucuucugguu

SEQ ID NO: 251 - RNA, 19 nt, Artificial Sequence
  siRNA
  modified_base, modified as per summary sequence table at the end of the description
aaccagaagaagcagguga

SEQ ID NO: 252 - RNA, 19 nt, Artificial Sequence
  siRNA
  modified_base, modified as per summary sequence table at the end of the description
ucaccugcuucuucugguu

SEQ ID NO: 253 - RNA, 19 nt, Artificial Sequence
  siRNA
  modified_base, modified as per summary sequence table at the end of the description
aaccagaagaagcagguga

SEQ ID NO: 254 - RNA, 19 nt, Artificial Sequence
  siRNA
  modified_base, modified as per summary sequence table at the end of the description
ucaccugcuucuucugguu

SEQ ID NO: 255 - RNA, 19 nt, Artificial Sequence
  siRNA
  modified_base, modified as per summary sequence table at the end of the description
aaccagaagaagcagguga

SEQ ID NO: 256 - RNA, 19 nt, Artificial Sequence
  siRNA
  modified_base, modified as per summary sequence table at the end of the description
ucaccugcuucuucugguu

SEQ ID NO: 257 - RNA, 19 nt, Artificial Sequence
  siRNA
  modified_base, modified as per summary sequence table at the end of the description
aaccagaagaagcagguga

SEQ ID NO: 258 - RNA, 19 nt, Artificial Sequence
  siRNA
  modified_base, modified as per summary sequence table at the end of the description
ucaccugcuucuucugguu

SEQ ID NO: 259 - RNA, 19 nt, Artificial Sequence
  siRNA
  modified_base, modified as per summary sequence table at the end of the description
aaccagaagaagcagguga

SEQ ID NO: 260 - RNA, 19 nt, Artificial Sequence
  siRNA
  modified_base, modified as per summary sequence table at the end of the description
ucaccugcuucuucugguu

SEQ ID NO: 261 - RNA, 19 nt, Artificial Sequence
  siRNA
  modified_base, modified as per summary sequence table at the end of the description
aaccagaagaagcagguga

SEQ ID NO: 262 - RNA, 19 nt, Artificial Sequence
  siRNA
  modified_base, modified as per summary sequence table at the end of the description
ucaccugcuucuucugguu

SEQ ID NO: 263 - RNA, 19 nt, Artificial Sequence
  siRNA
  modified_base, modified as per summary sequence table at the end of the description
aaccagaagaagcagguga

SEQ ID NO: 264 - RNA, 19 nt, Artificial Sequence
  siRNA
  modified_base, modified as per summary sequence table at the end of the description
ucaccugcuucuucugguu

SEQ ID NO: 265 - RNA, 19 nt, Artificial Sequence
  siRNA
  modified_base, modified as per summary sequence table at the end of the description
aaccagaagaagcagguga

SEQ ID NO: 266 - RNA, 19 nt, Artificial Sequence
  siRNA
  modified_base, modified as per summary sequence table at the end of the description
ucaccugcuucuucugguu

SEQ ID NO: 267 - RNA, 19 nt, Artificial Sequence
  siRNA
  modified_base, modified as per summary sequence table at the end of the description
aaccagaagaagcagguga

SEQ ID NO: 268 - RNA, 19 nt, Artificial Sequence
  siRNA
  modified_base, modified as per summary sequence table at the end of the description
ucaccugcuucuucugguu

SEQ ID NO: 269 - RNA, 19 nt, Artificial Sequence
  siRNA
  modified_base, modified as per summary sequence table at the end of the description
aaccagaagaagcagguga

SEQ ID NO: 270 - RNA, 19 nt, Artificial Sequence
  siRNA
  modified_base, modified as per summary sequence table at the end of the description
ucaccugcuucuucugguu

SEQ ID NO: 271 - RNA, 19 nt, Artificial Sequence
  siRNA
  modified_base, modified as per summary sequence table at the end of the description
aaccagaagaagcagguga

SEQ ID NO: 272 - RNA, 19 nt, Artificial Sequence
  siRNA
  modified_base, modified as per summary sequence table at the end of the description
ucaccugcuucuucugguu

SEQ ID NO: 273 - RNA, 19 nt, Artificial Sequence
  siRNA
  modified_base, modified as per summary sequence table at the end of the description
aaccagaagaagcagguga

SEQ ID NO: 274 - RNA, 19 nt, Artificial Sequence
  siRNA
  modified_base, modified as per summary sequence table at the end of the description
ucaccugcuucuucugguu

SEQ ID NO: 275 - RNA, 19 nt, Artificial Sequence
  siRNA
  modified_base, modified as per summary sequence table at the end of the description
aaccagaagaagcagguga

SEQ ID NO: 276 - RNA, 19 nt, Artificial Sequence
  siRNA
  modified_base, modified as per summary sequence table at the end of the description
ucaccugcuucuucugguu

SEQ ID NO: 277 - RNA, 19 nt, Artificial Sequence
  siRNA
  modified_base, modified as per summary sequence table at the end of the description
aaccagaagaagcagguga

SEQ ID NO: 278 - RNA, 19 nt, Artificial Sequence
  siRNA
  modified_base, modified as per summary sequence table at the end of the description
ucaccugcuucuucugguu

SEQ ID NO: 279 - RNA, 19 nt, Artificial Sequence
  siRNA
  modified_base, modified as per summary sequence table at the end of the description
aaccagaagaagcagguga

SEQ ID NO: 280 - RNA, 19 nt, Artificial Sequence
  siRNA
  modified_base, modified as per summary sequence table at the end of the description
ucaccugcuucuucugguu

SEQ ID NO: 281 - RNA, 19 nt, Artificial Sequence
  siRNA
  modified_base, modified as per summary sequence table at the end of the description
aaccagaagaagcagguga

SEQ ID NO: 282 - RNA, 19 nt, Artificial Sequence
  siRNA
  modified_base, modified as per summary sequence table at the end of the description
ucaccugcuucuucugguu

SEQ ID NO: 283 - RNA, 19 nt, Artificial Sequence
  siRNA
  modified_base, modified as per summary sequence table at the end of the description
aaccagaagaagcagguga

SEQ ID NO: 284 - RNA, 19 nt, Artificial Sequence
  siRNA
  modified_base, modified as per summary sequence table at the end of the description
ucaccugcuucuucugguu

SEQ ID NO: 285 - RNA, 19 nt, Artificial Sequence
  siRNA
  modified_base, modified as per summary sequence table at the end of the description
aaccagaagaagcagguga

SEQ ID NO: 286 - RNA, 19 nt, Artificial Sequence
  siRNA
  modified_base, modified as per summary sequence table at the end of the description
ucaccugcuucuucugguu

SEQ ID NO: 287 - RNA, 19 nt, Artificial Sequence
  siRNA
  modified_base, modified as per summary sequence table at the end of the description
aaccagaagaagcagguga

SEQ ID NO: 288 - RNA, 19 nt, Artificial Sequence
  siRNA
  modified_base, modified as per summary sequence table at the end of the description
ucaccugcuucuucugguu

SEQ ID NO: 289 - RNA, 19 nt, Artificial Sequence
  siRNA
  modified_base, modified as per summary sequence table at the end of the description
aaccagaagaagcagguga

SEQ ID NO: 290 - RNA, 19 nt, Artificial Sequence
  siRNA
  modified_base, modified as per summary sequence table at the end of the description
ucaccugcuucuucugguu

SEQ ID NO: 291 - RNA, 19 nt, Artificial Sequence
  siRNA
  modified_base, modified as per summary sequence table at the end of the description
aaccagaagaagcagguga

SEQ ID NO: 292 - RNA, 19 nt, Artificial Sequence
  siRNA
  modified_base, modified as per summary sequence table at the end of the description
ucaccugcuucuucugguu

SEQ ID NO: 293 - RNA, 19 nt, Artificial Sequence
  siRNA
  modified_base, modified as per summary sequence table at the end of the description
uaccagaagaagcagguga

SEQ ID NO: 294 - RNA, 19 nt, Artificial Sequence
  siRNA
  modified_base, modified as per summary sequence table at the end of the description
ucaccugcuucuucuggua

SEQ ID NO: 295 - RNA, 19 nt, Artificial Sequence
  siRNA
  modified_base, modified as per summary sequence table at the end of the description
uaccagaagaagcagguga

SEQ ID NO: 296 - RNA, 19 nt, Artificial Sequence
  siRNA
  modified_base, modified as per summary sequence table at the end of the description
ucaccugcuucuucuggua

SEQ ID NO: 297 - RNA, 19 nt, Artificial Sequence
  siRNA
  modified_base, modified as per summary sequence table at the end of the description
uaccagaagaagcagguga

SEQ ID NO: 298 - RNA, 19 nt, Artificial Sequence
  siRNA
  modified_base, modified as per summary sequence table at the end of the description
ucaccugcuucuucuggua

SEQ ID NO: 299 - RNA, 19 nt, Artificial Sequence
  siRNA
  modified_base, modified as per summary sequence table at the end of the description
uaccagaagaagcagguga

SEQ ID NO: 300 - RNA, 19 nt, Artificial Sequence
  siRNA
  modified_base, modified as per summary sequence table at the end of the description
ucaccugcuucuucuggua

SEQ ID NO: 301 - RNA, 19 nt, Artificial Sequence
  siRNA
  modified_base, modified as per summary sequence table at the end of the description
ucgaaguauuccgcguacg

SEQ ID NO: 302 - RNA, 19 nt, Artificial Sequence
  siRNA
  modified_base, modified as per summary sequence table at the end of the description
cguacgcggaauacuucga

SEQ ID NO: 303 - RNA, 22 nt, Artificial Sequence
  siRNA
  modified_base, modified as per summary sequence table at the end of the description
caccgccaaatttaactgcaga

SEQ ID NO: 304 - RNA, 24 nt, Artificial Sequence
  siRNA
  modified_base, modified as per summary sequence table at the end of the description
aagggtttgataagttctagctgt

SEQ ID NO: 305 - RNA, 31 nt, Artificial Sequence; identical to SEQ ID NO: 49
  siRNA
  modified_base, modified as per summary sequence table at the end of the description

SEQ ID NO: 306 - RNA, 17 nt, Artificial Sequence
  siRNA
  modified_base, modified as per summary sequence table at the end of the description
ccgccaaagcccagaag

SEQ ID NO: 307 - RNA, 21 nt, Artificial Sequence
  siRNA
  modified_base, modified as per summary sequence table at the end of the description
ggtccctccccaaaggaatag

SEQ ID NO: 308 - RNA, 28 nt, Artificial Sequence
  siRNA
  modified_base, modified as per summary sequence table at the end of the description
cagcacccgcctgggaacttactacaac

SEQ ID NO: 309 - RNA, 19 nt, Artificial Sequence
  siRNA
  modified_base, modified as per summary sequence table at the end of the description
aaccagaagaagcagguga

SEQ ID NO: 310 - RNA, 19 nt, Artificial Sequence
  siRNA
  modified_base, modified as per summary sequence table at the end of the description
ucaccugcuucuucugguu

SEQ ID NO: 311 - RNA, 19 nt, Artificial Sequence
  siRNA
  modified_base, modified as per summary sequence table at the end of the description
aaccagaagaagcagguga

SEQ ID NO: 312 - RNA, 19 nt, Artificial Sequence
  siRNA
  modified_base, modified as per summary sequence table at the end of the description
ucaccugcuucuucugguu

SEQ ID NO: 313 - RNA, 19 nt, Artificial Sequence
  siRNA
  modified_base, modified as per summary sequence table at the end of the description
aaccagaagaagcagguga

SEQ ID NO: 314 - RNA, 19 nt, Artificial Sequence
  siRNA
  modified_base, modified as per summary sequence table at the end of the description
ucaccugcuucuucugguu

SEQ ID NO: 315 - RNA, 19 nt, Artificial Sequence
  siRNA
  modified_base, modified as per summary sequence table at the end of the description
aaccagaagaagcagguga

SEQ ID NO: 316 - RNA, 19 nt, Artificial Sequence
  siRNA
  modified_base, modified as per summary sequence table at the end of the description
ucaccugcuucuucugguu

SEQ ID NO: 317 - RNA, 19 nt, Artificial Sequence
  siRNA
augucuuucacacuggcuu

SEQ ID NO: 318 - RNA, 19 nt, Artificial Sequence
  siRNA
aagccagugugaaagacau

SEQ ID NO: 319 - RNA, 19 nt, Artificial Sequence
  siRNA
auugaguacacgcagacug

SEQ ID NO: 320 - RNA, 19 nt, Artificial Sequence
  siRNA
cagucugcguguacucaau

SEQ ID NO: 321 - RNA, 19 nt, Artificial Sequence
  siRNA
aaguugauggugaucccgg

SEQ ID NO: 322 - RNA, 19 nt, Artificial Sequence
  siRNA
ccgggaucaccaucaacuu

SEQ ID NO: 323 - RNA, 19 nt, Artificial Sequence
  siRNA
uucuggaucguccacuggc

SEQ ID NO: 324 - RNA, 19 nt, Artificial Sequence
  siRNA
gccaguggacgauccagaa

SEQ ID NO: 325 - RNA, 19 nt, Artificial Sequence
  siRNA
auucacagaacagaggaac

SEQ ID NO: 326 - RNA, 19 nt, Artificial Sequence
  siRNA
guuccucuguucugugaau

SEQ ID NO: 327 - RNA, 19 nt, Artificial Sequence
  siRNA
guagucauggcuguccucu

SEQ ID NO: 328 - RNA, 19 nt, Artificial Sequence
  siRNA
agaggacagccaugacuac

SEQ ID NO: 329 - RNA, 19 nt, Artificial Sequence
  siRNA
aguuguaguaaguucccag

SEQ ID NO: 330 - RNA, 19 nt, Artificial Sequence
  siRNA
cugggaacuuacuacaacu

SEQ ID NO: 331 - RNA, 19 nt, Artificial Sequence
  siRNA
uuguacccuaggaaauacc

SEQ ID NO: 332 - RNA, 19 nt, Artificial Sequence
  siRNA
gguauuuccuaggguacaa

SEQ ID NO: 333 - RNA, 19 nt, Artificial Sequence
  siRNA
aaccagaagaagcagguga

SEQ ID NO: 334 - RNA, 19 nt, Artificial Sequence
  siRNA
ucaccugcuucuucugguu

SEQ ID NO: 335 - RNA, 19 nt, Artificial Sequence
  siRNA
uaacaacccagcguggaau

SEQ ID NO: 336 - RNA, 19 nt, Artificial Sequence
  siRNA
auuccacgcuggguuguua

SEQ ID NO: 337 - RNA, 19 nt, Artificial Sequence
  siRNA
guuucucucauccaggccg

SEQ ID NO: 338 - RNA, 19 nt, Artificial Sequence
  siRNA
cggccuggaugagagaaac

SEQ ID NO: 339 - RNA, 19 nt, Artificial Sequence
  siRNA
gcaucuucugggcuuuggc

SEQ ID NO: 340 - RNA, 19 nt, Artificial Sequence
  siRNA
gccaaagcccagaagaugc

SEQ ID NO: 341 - RNA, 19 nt, Artificial Sequence
  siRNA
ucacacuggaaggugaaug

SEQ ID NO: 342 - RNA, 19 nt, Artificial Sequence
  siRNA
cauucaccuuccaguguga

SEQ ID NO: 343 - RNA, 19 nt, Artificial Sequence
  siRNA
cacagaugugucgaccccg

SEQ ID NO: 344 - RNA, 19 nt, Artificial Sequence
  siRNA
cggggucgacacaucugug

SEQ ID NO: 345 - RNA, 19 nt, Artificial Sequence
  siRNA
uguacccuaggaaauacca

SEQ ID NO: 346 - RNA, 19 nt, Artificial Sequence
  siRNA
ugguauuuccuaggguaca

SEQ ID NO: 347 - RNA, 19 nt, Artificial Sequence
  siRNA
ucgaaguauuccgcguacg

SEQ ID NO: 348 - RNA, 19 nt, Artificial Sequence
  siRNA
cguacgcggaauacuucga

SEQ ID NO: 349 - RNA, 19 nt, Artificial Sequence
  siRNA
uaaguucuagcuguggugg

SEQ ID NO: 350 - RNA, 19 nt, Artificial Sequence
  siRNA
ccaccacagcuagaacuua

SEQ ID NO: 351 - RNA, 21 nt, Artificial Sequence
  siRNA
ucuugguuacaugaaauccca

SEQ ID NO: 352 - RNA, 21 nt, Artificial Sequence
  siRNA
ugggauuucauguaaccaaga

SEQ ID NO: 353 - RNA, 21 nt, Artificial Sequence
  siRNA
aaccagaagaagcaggugacc

SEQ ID NO: 354 - RNA, 19 nt, Artificial Sequence
  siRNA
uuaguaaaccuuuugagac

SEQ ID NO: 355 - RNA, 19 nt, Artificial Sequence
  siRNA
gucucaaaagguuuacuaa

SEQ ID NO: 356 - RNA, 19 nt, Artificial Sequence
  siRNA
cugaggacgcccugggagu

SEQ ID NO: 357 - RNA, 19 nt, Artificial Sequence
  siRNA
acucccagggcguccucag

SEQ ID NO: 358 - RNA, 19 nt, Artificial Sequence
  siRNA
gcugaggacgcccugggag

SEQ ID NO: 359 - RNA, 19 nt, Artificial Sequence
  siRNA
cucccagggcguccucagc

SEQ ID NO: 360 - RNA, 19 nt, Artificial Sequence
  siRNA
ugcugaggacgcccuggga

SEQ ID NO: 361 - RNA, 19 nt, Artificial Sequence
  siRNA
ucccagggcguccucagca

SEQ ID NO: 362 - RNA, 19 nt, Artificial Sequence
  siRNA
gugcugaggacgcccuggg

SEQ ID NO: 363 - RNA, 19 nt, Artificial Sequence
  siRNA
cccagggcguccucagcac

SEQ ID NO: 364 - RNA, 19 nt, Artificial Sequence
  siRNA
ggugcugaggacgcccugg

SEQ ID NO: 365 - RNA, 19 nt, Artificial Sequence
  siRNA
ccagggcguccucagcacc

SEQ ID NO: 366 - RNA, 19 nt, Artificial Sequence
  siRNA
gggugcugaggacgcccug

SEQ ID NO: 367 - RNA, 19 nt, Artificial Sequence
  siRNA
cagggcguccucagcaccc

SEQ ID NO: 368 - RNA, 19 nt, Artificial Sequence
  siRNA
cggggugcugaggacgccc

SEQ ID NO: 369 - RNA, 19 nt, Artificial Sequence
  siRNA
gggcguccucagcaccccg

SEQ ID NO: 370 - RNA, 19 nt, Artificial Sequence
  siRNA
acggggugcugaggacgcc

SEQ ID NO: 371 - RNA, 19 nt, Artificial Sequence
  siRNA
ggcguccucagcaccccgu

SEQ ID NO: 372 - RNA, 19 nt, Artificial Sequence
  siRNA
uacggggugcugaggacgc

SEQ ID NO: 373 - RNA, 19 nt, Artificial Sequence
  siRNA
gcguccucagcaccccgua

SEQ ID NO: 374 - RNA, 19 nt, Artificial Sequence
  siRNA
guacggggugcugaggacg

SEQ ID NO: 375 - RNA, 19 nt, Artificial Sequence
  siRNA
cguccucagcaccccguac

SEQ ID NO: 376 - RNA, 19 nt, Artificial Sequence
  siRNA
aguacggggugcugaggac

SEQ ID NO: 377 - RNA, 19 nt, Artificial Sequence
  siRNA
guccucagcaccccguacu

SEQ ID NO: 378 - RNA, 19 nt, Artificial Sequence
  siRNA
aaguacggggugcugagga

SEQ ID NO: 379 - RNA, 19 nt, Artificial Sequence
  siRNA
uccucagcaccccguacuu

SEQ ID NO: 380 - RNA, 19 nt, Artificial Sequence
  siRNA
ggaaguacggggugcugag

SEQ ID NO: 381 - RNA, 19 nt, Artificial Sequence
  siRNA
cucagcaccccguacuucc

SEQ ID NO: 382 - RNA, 19 nt, Artificial Sequence
  siRNA
gggaaguacggggugcuga

SEQ ID NO: 383 - RNA, 19 nt, Artificial Sequence
  siRNA
ucagcaccccguacuuccc

SEQ ID NO: 384 - RNA, 19 nt, Artificial Sequence
  siRNA
ggggaaguacggggugcug

SEQ ID NO: 385 - RNA, 19 nt, Artificial Sequence
  siRNA
cagcaccccguacuucccc

SEQ ID NO: 386 - RNA, 19 nt, Artificial Sequence
  siRNA
uggggaaguacggggugcu

SEQ ID NO: 387 - RNA, 19 nt, Artificial Sequence
  siRNA
agcaccccguacuucccca

SEQ ID NO: 388 - RNA, 19 nt, Artificial Sequence
  siRNA
cuggggaaguacggggugc

SEQ ID NO: 389 - RNA, 19 nt, Artificial Sequence
  siRNA
gcaccccguacuuccccag

SEQ ID NO: 390 - RNA, 19 nt, Artificial Sequence
  siRNA
agcuggggaaguacggggu

SEQ ID NO: 391 - RNA, 19 nt, Artificial Sequence
  siRNA
accccguacuuccccagcu

SEQ ID NO: 392 - RNA, 19 nt, Artificial Sequence
  siRNA
uagcuggggaaguacgggg

SEQ ID NO: 393 - RNA, 19 nt, Artificial Sequence
  siRNA
ccccguacuuccccagcua

SEQ ID NO: 394 - RNA, 19 nt, Artificial Sequence
  siRNA
guagcuggggaaguacggg

SEQ ID NO: 395 - RNA, 19 nt, Artificial Sequence
  siRNA
cccguacuuccccagcuac

SEQ ID NO: 396 - RNA, 19 nt, Artificial Sequence
  siRNA
aguagcuggggaaguacgg

SEQ ID NO: 397 - RNA, 19 nt, Artificial Sequence
  siRNA
ccguacuuccccagcuacu

SEQ ID NO: 398 - RNA, 19 nt, Artificial Sequence
  siRNA
guaguagcuggggaaguac

SEQ ID NO: 399 - RNA, 19 nt, Artificial Sequence
  siRNA
guacuuccccagcuacuac

SEQ ID NO: 400 - RNA, 19 nt, Artificial Sequence
  siRNA
aguaguagcuggggaagua

SEQ ID NO: 401 - RNA, 19 nt, Artificial Sequence
  siRNA
uacuuccccagcuacuacu

SEQ ID NO: 402 - RNA, 19 nt, Artificial Sequence
  siRNA
gaguaguagcuggggaagu

SEQ ID NO: 403 - RNA, 19 nt, Artificial Sequence
  siRNA
acuuccccagcuacuacuc

SEQ ID NO: 404 - RNA, 19 nt, Artificial Sequence
  siRNA
cgaguaguagcuggggaag

SEQ ID NO: 405 - RNA, 19 nt, Artificial Sequence
  siRNA
cuuccccagcuacuacucg

SEQ ID NO: 406 - RNA, 19 nt, Artificial Sequence
  siRNA
gcgaguaguagcuggggaa

SEQ ID NO: 407 - RNA, 19 nt, Artificial Sequence
  siRNA
uuccccagcuacuacucgc

SEQ ID NO: 408 - RNA, 19 nt, Artificial Sequence
  siRNA
ggcgaguaguagcugggga

SEQ ID NO: 409 - RNA, 19 nt, Artificial Sequence
  siRNA
uccccagcuacuacucgcc

SEQ ID NO: 410 - RNA, 19 nt, Artificial Sequence
  siRNA
gggcgaguaguagcugggg

SEQ ID NO: 411 - RNA, 19 nt, Artificial Sequence
  siRNA
ccccagcuacuacucgccc

SEQ ID NO: 412 - RNA, 19 nt, Artificial Sequence
  siRNA
ggggcgaguaguagcuggg

SEQ ID NO: 413 - RNA, 19 nt, Artificial Sequence
  siRNA
cccagcuacuacucgcccc

SEQ ID NO: 414 - RNA, 19 nt, Artificial Sequence
  siRNA
uggggcgaguaguagcugg

SEQ ID NO: 415 - RNA, 19 nt, Artificial Sequence
  siRNA
ccagcuacuacucgcccca

SEQ ID NO: 416 - RNA, 19 nt, Artificial Sequence
  siRNA
uuggggcgaguaguagcug

SEQ ID NO: 417 - RNA, 19 nt, Artificial Sequence
  siRNA
cagcuacuacucgccccaa

SEQ ID NO: 418 - RNA, 19 nt, Artificial Sequence
  siRNA
uauuccaaagggcagcuga

SEQ ID NO: 419 - RNA, 19 nt, Artificial Sequence
  siRNA
ucagcugcccuuuggaaua

SEQ ID NO: 420 - RNA, 19 nt, Artificial Sequence
  siRNA
aucuucugggcuuuggcgg

SEQ ID NO: 421 - RNA, 19 nt, Artificial Sequence
  siRNA
ccgccaaagcccagaagau

SEQ ID NO: 422 - RNA, 19 nt, Artificial Sequence
  siRNA
uuuucucuuggaguccuca

SEQ ID NO: 423 - RNA, 19 nt, Artificial Sequence
  siRNA
ugaggacuccaagagaaaa

SEQ ID NO: 424 - RNA, 19 nt, Artificial Sequence
  siRNA
gaauagacggagcuggagu

SEQ ID NO: 425 - RNA, 19 nt, Artificial Sequence
  siRNA
acuccagcuccgucuauuc

SEQ ID NO: 426 - RNA, 19 nt, Artificial Sequence
  siRNA
uaguagcuggggaaguacg

SEQ ID NO: 427 - RNA, 19 nt, Artificial Sequence
  siRNA
cguacuuccccagcuacua

SEQ ID NO: 428 - RNA, 19 nt, Artificial Sequence
  siRNA
agauccugggagaaguggc

SEQ ID NO: 429 - RNA, 19 nt, Artificial Sequence
  siRNA
gccacuucucccaggaucu

SEQ ID NO: 430 - RNA, 19 nt, Artificial Sequence
  siRNA
cuguucuggaucguccacu

SEQ ID NO: 431 - RNA, 19 nt, Artificial Sequence
  siRNA
aguggacgauccagaacag

SEQ ID NO: 432 - RNA, 19 nt, Artificial Sequence
  siRNA
cucaccuugaaggacaccu

SEQ ID NO: 433 - RNA, 19 nt, Artificial Sequence
  siRNA
agguguccuucaaggugag

SEQ ID NO: 434 - RNA, 19 nt, Artificial Sequence
  siRNA
aguuucucucauccaggcc

SEQ ID NO: 435 - RNA, 19 nt, Artificial Sequence
  siRNA
ggccuggaugagagaaacu

SEQ ID NO: 436 - RNA, 19 nt, Artificial Sequence
  siRNA
guacccuaggaaauaccag

SEQ ID NO: 437 - RNA, 19 nt, Artificial Sequence
  siRNA
cugguauuuccuaggguac

SEQ ID NO: 438 - RNA, 19 nt, Artificial Sequence
  siRNA
cuguugacuguggacagca

SEQ ID NO: 439 - RNA, 19 nt, Artificial Sequence
  siRNA
ugcuguccacagucaacag

SEQ ID NO: 440 - RNA, 19 nt, Artificial Sequence
  siRNA
uaccagaagaagcagguga

SEQ ID NO: 441 - RNA, 19 nt, Artificial Sequence
  siRNA
ucaccugcuucuucuggua

SEQ ID NO: 442 - RNA, 19 nt, Artificial Sequence
  siRNA
ucgaaguauuccgcguacg

SEQ ID NO: 443 - RNA, 19 nt, Artificial Sequence
  siRNA
cguacgcggaauacuucga

SEQ ID NO: 444 - RNA, 22 nt, Artificial Sequence
  siRNA
caccgccaaatttaactgcaga

SEQ ID NO: 445 - RNA, 24 nt, Artificial Sequence
  siRNA
aagggtttgataagttctagctgt

SEQ ID NO: 446 - RNA, 31 nt, Artificial Sequence; identical to SEQ ID NO: 49
  siRNA

SEQ ID NO: 447 - RNA, 17 nt, Artificial Sequence
  siRNA
ccgccaaagcccagaag

SEQ ID NO: 448 - RNA, 21 nt, Artificial Sequence
  siRNA
ggtccctccccaaaggaatag

SEQ ID NO: 449 - RNA, 28 nt, Artificial Sequence
  siRNA
cagcacccgcctgggaacttactacaac